European Patent Specification EP 3 978 624 B1, published March 26, 2025. Title: METHYLATED CONTROL DNA. Applicant: EXACT SCIENCES DEVELOPMENT COMPANY, LLC. Application EP. The sequence listing filed with the application follows.

SEQUENCE LISTING (13 sequences)

SEQ ID NO: 1 - DNA, 139 bp, Homo sapiens
ggccacacaggcccactctggccctctgagcccccggcggacccagggcattcaaggagcggctctgggctgccagcgcaggcctccgcgcaaacacagcaggctggaagtggcgctcatcaccggcacgtcttcccag

SEQ ID NO: 2 - DNA, 139 bp, Homo sapiens
ggttatataggtttattttggttttttgagttttcggcggatttagggtatttaaggagcggttttgggttgttagcgtaggttttcgcgtaaatatagtaggttggaagtggcgtttattatcggtacgtttttttag

SEQ ID NO: 3 - DNA, 28 bp, ArtIficial sequence
  Synthetic
ggtttattttggttttttgagttttcgg

SEQ ID NO: 4 - DNA, 24 bp, Artificial sequence
  Synthetic
tccaacctactatatttacgcgaa

SEQ ID NO: 5 - DNA, 21 bp, Artificial sequence
  Synthetic
gacgcggaggcggatttaggg

SEQ ID NO: 6 - DNA, 21 bp, Artificial sequence
  Synthetic
ccacggacggcggatttaggg

SEQ ID NO: 7 - DNA, 224 bp, Homo sapiens
ctctgacctgagtctcctttggaactctgcaggttctatttgctttttcccagatgagctctttttctggtgtttgtctctctgactaggtgtctaagacagtgttgtgggtgtaggtactaacactggctcgtgtgacaaggccatgaggctggtgtaaagcggccttggagtgtgtattaagtaggtgcacagtaggtctgaacagactccccatcccaaga

SEQ ID NO: 8 - DNA, 224 bp, Homo sapiens
ttttgatttgagttttttttggaattttgtaggttttatttgtttttttttagatgagttttttttttggtgtttgtttttttgattaggtgtttaagatagtgttgtgggtgtaggtattaatattggtttgtgtgataaggttatgaggttggtgtaaagtggttttggagtgtgtattaagtaggtgtatagtaggtttgaatagattttttattttaaga

SEQ ID NO: 9 - DNA, 30 bp, Artificial sequence
  Synthetic
gtgtttgtttttttgattaggtgtttaaga

SEQ ID NO: 10 - DNA, 26 bp, Artificial sequence
  Synthetic
ctttacaccaacctcataaccttatc

SEQ ID NO: 11 - DNA, 21 bp, Artificial sequence
  Synthetic
gacgcggagatagtgttgtgg

SEQ ID NO: 12 - DNA, 29 bp, Artificial sequence
  Synthetic
agccggttttccggctgagactccgcgtc

SEQ ID NO: 13 - DNA, 29 bp, Artificial sequence
  Synthetic
agccggttttccggctgagacgtccgtgg